European Patent Specification EP 3 965 813 B1, published November 20, 2024. Title: A NOVEL ORTHOBUNYAVIRUS IN HUMAN ENCEPHALITIS AND ITS DIAGNOSTIC AND THERAPEUTIC APPLICATIONS. Applicant: INSTITUT PASTEUR. The sequence listing filed with the application follows.

SEQUENCE LISTING (97 sequences)

SEQ ID NO: 1 - DNA, 772 bp, Moissiacense virus (Umbre orthobunyavirus strain Moissiacense)
  CDS (59)..(772)
aatcattatatctaaatttgctaaacgcagaactgggtagcactagcatttatccaggatggctgattctaagctcacatacgaggatacacaggatgttagtagaagtacttataacccagcagatgaatacgatacgtttgtgggtgtctacagagaatttctcacaattgataacattagaatcttcttcatcaacgctccaaaggccaaaactgcgatggctaaactcaagaccgagacagttgaagttacatttggaacactcgttgtcaagctggttaataaccatagaattggacaggctcagcgtgaggttgcggacgatgagctaactcttcaccgactttctggctacattgcaaagtacactcttcacctatacaaaaatgcaaaaaaagcaggagagagagaagcaataataaccaagatcgttaatccaatttctgccaaaatgggcttccaatggagtgttgggccggaaatttatctctcaacgctgccaggaaccgaaatgtttctagatacatttaaaatgttcccattggcattcatcttgttaagagttaaaagaggagagatcaaggtggaaatggcaaaaaaagcaatgcggcagaagtatggcgacaaagatgccagtgaatggctgcaggaggacattgagactgtaaaaggggcaataaaaacagttgaaaagctcaagccaacgctgacaggattggctgcttcaatgactgctttcctgcaacaacttggtatcaacactaagtaa

SEQ ID NO: 2 - protein, 237 aa, Moissiacense virus (Umbre orthobunyavirus strain Moissiacense)
MADSKLTYEDTQDVSRSTYNPADEYDTFVGVYREFLTIDNIRIFFINAPKAKTAMAKLKTETVEVTFGTLVVKLVNNHRIGQAQREVADDELTLHRLSGYIAKYTLHLYKNAKKAGEREAIITKIVNPISAKMGFQWSVGPEIYLSTLPGTEMFLDTFKMFPLAFILLRVKRGEIKVEMAKKAMRQKYGDKDASEWLQEDIETVKGAIKTVEKLKPTLTGLAASMTAFLQQLGINTK

SEQ ID NO: 3 - DNA, 4395 bp, Moissiacense virus (Umbre orthobunyavirus strain Moissiacense)
  CDS (1)..(4395)
  variation (4114)..(4116): nnn is att or aaa
atggtgatctttgcattgttgtcgatactattagttggcttcagcaatcaagcgactattcgatgtttctctggcggctccaaaatcatggaaaaaacatcgaatgtctcattgagtgaactatgcttaaaggatgatgtcagccagctaaaaattatagttgaccacacaaaaaatgattcaggattattttcaactgccagcgtctggagaaaatggatagtctcagattggaccacatgtaaccctaaaaaaatggctttaggaacaatatctgttatagatatcgataaaaactttatcttaaaaagctccagctatatatgcaataaagagtgcacgataacagtggataaagaaagagcccaagttctgctacaatcagatggcttaaatcactttgaagtttctggaaccactttgagttctggatggtttaaatcgacagccactgttaccttagatcaaacctgcgagcatgttaaagtgtcttgtggccagaaatcaatgcaattccatgcctgcttcaagaatcatatgtcatgcattagattcttgcatagaagtataatgccagcaagctttgcagtttctatctgccagaatatagagttgatattaatgacaacgtttacattgattatattcttgctactaagcattttaacaaaaacatacatatgctatattttgctacccatattcataccctttgcgtacgcatatggatttgtttatgataaaacatgcaagaagtgctcattatgtggattagcttaccaccctttcacaaagtgtgggatacattgtgtttgtggatgtagatttgaaaattcagatgcaatgaaaacccacagagaaaaagggaaatgtccgggattcaagtcaatgagaattgctagggtactgtgtaaggctaaaggttcagctttcgctttatctgtactattggccacgttggcattgggcttcttgacgcctgtacaagggctagttctagataagacccaaattaactacacagaagatcaattaccagaatcatttcagacgatgcaatcaacaatatctatattcaaatttgcaacagtcatgaatgcaggttggacttactgcatgttccttgttacattggctttatatatcatacacaagaagtatgctcacagattactgagctattatgtaatacattgcagggagtgtgacatgcttcatgacaaaagtgggcttaagtataatggtgattttactaacaaatgcggtttttgtacatgtgggcaagttgaagatgcaatggggctgaccgtccatcaaatacgaaatcattgctctgccaactatagaactaagatggtgctgaactggatgatcgtgctattattagctactctaatcaaagatagcataatgctgactgccgcagcagggacagaatttgaaacatgcatcaagaaagtagaaatgacaccggaatgcacaggacctttcatggaagttggaatctgtgatcaccagcagaagagcctaagataccatgagatagctaatatgttattgggtaaagggacaatctcaaaattagatgtggatattatagatgcattgcctgacaggatagctggagacctccagataatacagtcaagcagtgatttccaccatcaacagatgctggaatatgtgtttctattgcgtcattgtgattattactcaagttttgtttcggataacagctactcacaaatcttgtggcaaacagcagcaaagttaaatgaaaccaacctttgcaaacatgagaattcaaagaaatcctgcaagtgcttaaaatcaaatgcaaattgtggagagtcagaagacatcaacatagcagcacaggcatactacaaaaataaggaatctgagctaggacaagatctaacaaccataatgtacatactcaaaaaaatgattccaggatcaggttatagttatctgctaaatgcagccaagcacaacaaattagaattgttcaaagcttacatgactaatatttcctcaaaatattcaaataacaaaaaattaaaagatttcatggcgataataaatgctatactagcaaatctgtcagctctctcacatagtagtgaagaatcaatctcacaatacaaacagattgatttttcttccctagtaggcgaaacaacagacatgctcgaagcaaattttaatcaaacgatcagtacagacaagataatttgtgaaaatcctaaagtaatgatttgcatttcacccaggacaaaagtttcatccggtgaattgtatgtctgccaaagatcaggaaagtactacataatagataccggcaaattcaagctatataaattaattgacgcagacaatttgtactgtgcagcagatgctcagtgtaggtatgaatttagaattttaaccacaggggaaatgcaggcaacttttaaagataattgcaaagcatcagtacatgttaacaccccaggataccaaaatgaagctataactcattgcaaagtgctcgcgaatggtaaatgtaagtataataatcaaacttcaatagatataacattgtgtgctaacaacagatattatcccgaagcaaaaggcaggatctttggagttgatccagaagatctatgctttgataagacatgtactaaacaacagactccatacaacgaagaactaatcagtatgtgtgtttgggaaaatccgacacttaggccaatcaaacccagaactgaggtttctatgactttccaagagtacaaagatcagttattaaagaaaatcaacacagacctggtgctgcacaaatttgttagaacacaaaacttaccttatttcataccgcaattcaagtatataactatacaaggaacgtcaacaacagacgggattacttccagttttatattctttgaaattcctgcattgacaggagcatctgctggatacaaagttataaatagcgaaggccaagaattgatggacatggtagtttatatcaaaacatcaaagactagcgcaaagtacaagcgcgtgtattatacaggccccactatagctataaatacaaaacatcaagagcactgcacagggacatgtcctgaaagaatagaacatgatgaaggttgggcaacattttcgaaagaaagaaccagcaattggggctgtgaagaatttggttgtctagctgttgagactggttgtttatttgggtcatgccaggatgtaattagaagagaacttgatgttttttcaaagttggaggaagataaaatattgactgaactctgtataacattaagccatgacacttactgcgtgacaatcgattctacaacaccaacaatcaatgattactttgaaatccaatacaaaacagtagatgtacaaacattgccaaagatgataggagtcactcatcataagctattgcgagggcagataaacgaattaggatcatttggcaaattttgtggcaacatacaagtagttggtaatcaaacatatgggcaggctgcagtaaagtttgattacatttgccatgctgcacaaagaaaagatgtagttataagaaagtgcttagaaaataattaccaaagttgtaagctactgacacatgacacagacttgatacttgaagaaagtaagaccagtgttgaagtcataaacaataaaaggattacaggacaaatagcactaaaggtcttgttgggagactttaactacaagcagtatgctgcaaatgtagaggctgacatagaagcaaattgcgttgggtgtacaaattgtataaagggaataacatgtgaaataaaggtgaaaacagaaattgaagcatcatgtaaggtagagcccccatgcccctcttacacaagtagaattataataaaaccaggtagagacacccacacattattgatgaagtgtgacaaaaaaataacgactggtgaactagcaataaaaatatgtaatatgcaaatccaggctcatctttcaacaatagagagcaatgaccaactagaattgtcgactggggatcaatcaacatatatacatgaagaagacctaaggtgttcaacctggatctgcawwgtgagagacgaagggataagcttcatctttaagccattaacagactggcttggaagcttcacaaagccgatacttatagctggctgtatgataattgttgcaattattttgatttatatattaatgcctatgtgtgctagactcagagatttgttaaagaaaaacgagtatgaatatctacaagatacaaaagtgattgtaaagcccaagggtacagcaagttcaataggcttgagatcgaagaaaataaatatccaatcgtctaaggctgttgattaa

SEQ ID NO: 4 - protein, 1464 aa, Moissiacense virus (Umbre orthobunyavirus strain Moissiacense)
  misc_feature (1372)..(1372): The 'Xaa' at location 1372 stands for Lys, Asn, or Ile.
MVIFALLSILLVGFSNQATIRCFSGGSKIMEKTSNVSLSELCLKDDVSQLKIIVDHTKNDSGLFSTASVWRKWIVSDWTTCNPKKMALGTISVIDIDKNFILKSSSYICNKECTITVDKERAQVLLQSDGLNHFEVSGTTLSSGWFKSTATVTLDQTCEHVKVSCGQKSMQFHACFKNHMSCIRFLHRSIMPASFAVSICQNIELILMTTFTLIIFLLLSILTKTYICYILLPIFIPFAYAYGFVYDKTCKKCSLCGLAYHPFTKCGIHCVCGCRFENSDAMKTHREKGKCPGFKSMRIARVLCKAKGSAFALSVLLATLALGFLTPVQGLVLDKTQINYTEDQLPESFQTMQSTISIFKFATVMNAGWTYCMFLVTLALYIIHKKYAHRLLSYYVIHCRECDMLHDKSGLKYNGDFTNKCGFCTCGQVEDAMGLTVHQIRNHCSANYRTKMVLNWMIVLLLATLIKDSIMLTAAAGTEFETCIKKVEMTPECTGPFMEVGICDHQQKSLRYHEIANMLLGKGTISKLDVDIIDALPDRIAGDLQIIQSSSDFHHQQMLEYVFLLRHCDYYSSFVSDNSYSQILWQTAAKLNETNLCKHENSKKSCKCLKSNANCGESEDINIAAQAYYKNKESELGQDLTTIMYILKKMIPGSGYSYLLNAAKHNKLELFKAYMTNISSKYSNNKKLKDFMAIINAILANLSALSHSSEESISQYKQIDFSSLVGETTDMLEANFNQTISTDKIICENPKVMICISPRTKVSSGELYVCQRSGKYYIIDTGKFKLYKLIDADNLYCAADAQCRYEFRILTTGEMQATFKDNCKASVHVNTPGYQNEAITHCKVLANGKCKYNNQTSIDITLCANNRYYPEAKGRIFGVDPEDLCFDKTCTKQQTPYNEELISMCVWENPTLRPIKPRTEVSMTFQEYKDQLLKKINTDLVLHKFVRTQNLPYFIPQFKYITIQGTSTTDGITSSFIFFEIPALTGASAGYKVINSEGQELMDMVVYIKTSKTSAKYKRVYYTGPTIAINTKHQEHCTGTCPERIEHDEGWATFSKERTSNWGCEEFGCLAVETGCLFGSCQDVIRRELDVFSKLEEDKILTELCITLSHDTYCVTIDSTTPTINDYFEIQYKTVDVQTLPKMIGVTHHKLLRGQINELGSFGKFCGNIQVVGNQTYGQAAVKFDYICHAAQRKDVVIRKCLENNYQSCKLLTHDTDLILEESKTSVEVINNKRITGQIALKVLLGDFNYKQYAANVEADIEANCVGCTNCIKGITCEIKVKTEIEASCKVEPPCPSYTSRIIIKPGRDTHTLLMKCDKKITTGELAIKICNMQIQAHLSTIESNDQLELSTGDQSTYIHEEDLRCSTWICXVRDEGISFIFKPLTDWLGSFTKPILIAGCMIIVAIILIYILMPMCARLRDLLKKNEYEYLQDTKVIVKPKGTASSIGLRSKKINIQSSKAVD

SEQ ID NO: 5 - DNA, 6828 bp, Moissiacense virus (Umbre orthobunyavirus strain Moissiasence)
  CDS (1)..(6828)
atgctggaccaagaaaatgagcaagctttaaatagacttgcagccgcagttgcgagagcaaatgagcctgccgaaggcaaagaagcatataatgctatactgagtagaaggcatgattactttgggcaagttttttgtgagaccataggcataccatacaggaacgatgttcggctagaggatatcctacatgaatgtgaccaaacagtcgacactctaacaaataagataccaaacataactccagacaactttgagtttagagacaatatcctaactataatagattataaagtagcagttagtgatgaaagtgctgactatactcgtgaaaagtatgaaaatgctgttgatgccataaagcatttggttgactttcctattagagtgtgtatagttaggatacacccatacactagacaagttacttactctgatgacaattttatgagacgatttgcccatgtggtataccctgttgattttacaaggtatactcaattaactgaagaactcaaggaaaaatttgcagatagccctgaatttatggatatgatagcatatggcgatgtcacttttactgcaaactggtgtcaaaatggatgccctgagctatatgggcatccgatattcaaagaatttttagaaagcatgccattgaaataccagaaattgtttgaaaagtctttactgagttcttgctatacttctgagagatgggattccaatcttaaagaagtcaagggtgcaactaaagatgagtatgaagattttatatctcgatctgcaagagagctctatacaacatctcctgactattcagaacctagtcgagaggaaattctaaaagggtgggaagaaatgacagaacgagtgaaagaacaaagggaagtgtcctcaaatattaatgaccaaaagccaagtgctcacttcatatgggctgaaaacaatcctgaactaccgactgcaaattctgctaagatatgtgcaatttcaaaacttttacagtccattaacatagaaagctcttttgctgaggattttaaaagactaggcaaattattcgacttttctgaagatatccctggatatgagcgacattgcgaacaacttaaaaggcaggctagatcaaatccaggacaaataaaaaacaaaaaactagacccaaagaaaattgggaatgcattagttttatgggagcaacaatttttattatctgcagatgaaatggggaaagagaataaactacacttacttaaagacttctttggcatagggaaacacaaacaatttgcaaaaaaaggcttagatgacactgaaacagataaaccgacaatcttagattttaatgatacagaagtcaaaagatcagcagagttgatgatgcaaagaacaaaactctacttatctggcaggtcgtcactcaataaagaacatcctgtagcatcagaatatctaaatgaaataaaaaagtgtaatgatgagacacataatgttctgaatgcaatctttcagacaaaatattggcaatgtatcacagatattagcatgctaatgaaaaatatgctttctgtgtcgcagtataatagaaacaatactttcagaattgcaacatgtgctaataatgcactatatggacttatctttccgtcggcagatattaaaacaaaggatgcaagcattgtatattgcattattgcaattcataaagatgagaagtctttattcaatccaggagctctacatgcaactttcaaagtgccaggtggctttttatctatatctaaatcaatgcgacttgacaagaagcgctgtcacagaatagttactagtccaggcatattcttaacaattgccaccatgttgaaaggagataatccaactattagtttgaatgatgttttaaattttagcatttttgcgagcttgaacataactaagagcatgctatcattaacagagccttctaggtatatgatcatgaactcattagcagtctccagtcatgtacgcgaatacatctctgagaaattttcgccatatactaaaactctctttagtgtccatatggttgagaaaataaaagcaggctgtctaaatgcattcaaacaaagagaaaaaatcaagactcgcgacatatacttgacagacatagatataactcaaaaagggatacaagataacagagacctatgtagcatatggtttgatggtaatgtcactttgaaagaatatctaaaccagatttatattgtcttttatctgaatccaaaagcattacatgaaaagcatcatgtaatgatagatttactcaaaacagtgatagaaatagaactcgatcaaagggagaatgtccctcaaccatggtctgacgtcccaaaaaagcagactgtcaatttgcccattcttgttcatagcctagcaaagaatctacttctagacacttcattcgcgcatttcttaaggtctagaattgaaagccgcaataattttagacgcacgtttgcaacaatttcaacttttacaagtagtaagagttgcttaaaaacaggcaatttccatgagttcaagattaagcaatgtcaacggctcaaaaaagtgaatacaagtgaagcaaaaaaacatagaatagcaaatgccatgtttgttgaggaacaagaccaacatttagaggtggagcatgcaaactacgaattaatgaggaaggcaatcccggattatgtggatgtcttatcgaccaaagtattcgatagattatatgagctatataaaactggagagattgatgacagtcctgttatccatcagatttttgcgaccatgaaaagccacactaaattctattttacttattttaataaaggccaaaaaacagcaaaagaccgagaaatatttgtaggggaatacgaggccaaaatgtgtatgtatctggtagaaagaatatataaagagagatcgaaagtcaatccagacgaaatgatcagtgaaccaggagatgggaaactcagagtgctagagcgcaaagcagagcaagagataagattcatggttgaaaaaatgaaagcaaagaatgatgaaataaataaggaaatcgaggatgcaaaagacaattatgtcctaaatttagggaaaatagcagcactgcaagcacaaaaatataaagctttaaaattggaaatcaatgcagacatgtcaaagtggagtgctcaagacgtgttctttaaatacttttggtctgtctgtcttgacccaattctctatcctgaagaaaaagaacacattttatattttttttgtaactatatgcaaaaagaattggttatcccagatgaggttatctgcaatatcctagatcagaggaaagcataccctaatgacataattagtcagatcacaaatggcttgacaaccaaccatttcaatgtaaagagaaactggctacaaggcaacttcaattacatgtccagctatgctcacagtacagcaatgtctgtctttaaagatgtgataaagcgtgctgcagatttactagaagctgaagttctgattcattctatggttcactctgatgataaccagacctctgtaacattggtcgacaacaggatatgcccaaagcaattcacagcatttgtaatcaatacatttgaaaagatctgcctaacattcggctgtcaagctaatatgaaaaaaacctatatcaccaaccatataaaagaatttgtttcactattcaatttatatggagaaccattttcaatttatggcagattcacattaacatctgttggagactgcgcatacatcggaccatacgaagatctcgcaagcaggatatcagcaacacaaaccgggataaagcatggatgcccagctagccaagcctggttatcgattactatcgcccaatggatgacttacttgacatataatatgttgccaggccaacaaaatgacccctggccaatattggaaatcgatagaaagcaattgccacttgagttgggtggatacatctcttgtcctctatccttaatagctttagctgggctagaatccgggaacattgatttcctgatcaaattggtaaacaaatatgttgaccccagacttcaacgtgaacctatccaggatcaatgcactgatataaaaaactgggacatttcaaggcttagcaaagttgaaatatttaagctaaaagtgctgcgttatttagttttagatgcagagatggataatactgacattatgggagaaaccagcgaaatgagaggaagatccttactaacacccaggaagttcacaacagctggctccttgagaaaattggtatcttttgaagatttccaagcggtgcaagatactgaacaaggtgtggatgttatagttgagtacatgctgcaaaacccagcattgctcgtgacaaagggagaaacaaaagatgactatatgaacacagtgctctatagatataactcaaagaaatttaaagaatcattatccattcagaatcctactcagctctttttggagcaaatcctattctctcacaagcctattgttgattatacaggtatcgcagaaaagttctcaaatcttaatgatggaaccatgcttgaagataatccgacaataaaaggtaggatgacctttacagatgctttcgcaatgatcaagaaagatctatcaacactcaaaatcaccaatgaggaccttgaaattgtgctaaaatttataattttgaatgaccctttgactgtgactgctgccaacgcccatatcttgcatgtaataggtcattcacaacctaggcttggatcaacagcttgtgttatgcctgaatttaggaatttgagaatgataaaacattcacctgcactagtcttaaagtgttatagtaaaaacactttgttgctgcccggggtgcaagaaagagacatggaaagggaccttaaccatctcaaaacatttattgagactacaagattagagcataaaatgcaagataggatcaagaaaaatgaagatctcaaaaaatcgaaggatatctactttgaaatcaaagaggtaactagattttatcaaacatgctatgaatatgtcaaaagtactgattataaggtaaaagtattcatactaccagccaaatgtatgactcaaacagatttttgcgctgtattacagggttcattgttagaagataaaaagtggaaattaatacaacacctcagacctgttactgcaggtggacataaaggagaggttcagccggtagtttccatggattttaaactagcaagagaggccgtaaatttattatgcttttttactgattcatttatagactctagatatagaagagactttcttctaaaagcgtgcgtagaaatggcttataaagataggcctatggttacattgatagaagaaataaagaagtcaaagaaccgaacatctttcttgccattcttgtatagaattggagagttaactcaagaagacctagatgcatatgatgctcaaaaagcgggagggagagtaacctggaatcactggcaatctacaagaagcttaaacatggggaagatagatttccaaatagatacacataaaagtcatctccatattattggagaagatcaacaattagtaatagcagagctaaaaattcctaaattgacagcaaatgctatcactcaagcaggatatagacttttaaatgaaaagcatgggtttcggtttgaaacaatgaatgaggttttagtccagccaagaaaatattatataacataccagatgaaatctaaaaagcaatatgtctataaaatctttgacacagcaacattgctatatgaaagaagaaacataaagcaatacacaggccgagaagcaaatcccatagtagcagtctgcgaagttgttccaatggaggaggaggaaactcccgctttaagcttaagtgacatagaaatgtataatgctgacaatgaatcagttagcattttaaaaacttcattcaatgagagtgcgaagatgagacgtgcaaatttgtccaaaatgcaatattttgagactattggcggatcaatgttgaaaattcgattcatcaatgtcaacgcactaatgaaagacacaactctaatgtcccttaactatgacaatttggtaaatgtcgacctggctagatttagcaagttattggactgtgacggtgatacagaaagtgttgaagatggaatattgtgcttttctgatgacccaatggaacaaaccacaacagaagagattgacgcgatccctctcttcaaagtaagctacaagatacctacaccagctagattaacatacaagaatgccattagagaactgttaaggagggaaataacaaggtttatggatgcttttacctttgttggaccttcttttgattcaccagaaaatatggggttcatatgcaatatatgttgtataatacaactcctccatacaaacgaatggtctactataatgctaaattgtattcatatctgcatgatttatctggagaaagacataaggtttcataaatttttactaaatagaatattctttgagggattgaatcctgcatctgggaaattggattacaaaaaaatcaaagaatttgtaatcagcctgaaggatagagagatggctccttggaatgagatattttcaaagttcaagcaaaaatgtgtcacattgctagacaaagaaataacaagaatagaacaaaacacaaactttgaaaatatactagctttagatgaaagcacagatgatcagtctggattcctcttgtttgaatag

SEQ ID NO: 6 - protein, 2275 aa, Moissiacense virus (Umbre orthobunyavirus strain Moissiasence)
MLDQENEQALNRLAAAVARANEPAEGKEAYNAILSRRHDYFGQVFCETIGIPYRNDVRLEDILHECDQTVDTLTNKIPNITPDNFEFRDNILTIIDYKVAVSDESADYTREKYENAVDAIKHLVDFPIRVCIVRIHPYTRQVTYSDDNFMRRFAHVVYPVDFTRYTQLTEELKEKFADSPEFMDMIAYGDVTFTANWCQNGCPELYGHPIFKEFLESMPLKYQKLFEKSLLSSCYTSERWDSNLKEVKGATKDEYEDFISRSARELYTTSPDYSEPSREEILKGWEEMTERVKEQREVSSNINDQKPSAHFIWAENNPELPTANSAKICAISKLLQSINIESSFAEDFKRLGKLFDFSEDIPGYERHCEQLKRQARSNPGQIKNKKLDPKKIGNALVLWEQQFLLSADEMGKENKLHLLKDFFGIGKHKQFAKKGLDDTETDKPTILDFNDTEVKRSAELMMQRTKLYLSGRSSLNKEHPVASEYLNEIKKCNDETHNVLNAIFQTKYWQCITDISMLMKNMLSVSQYNRNNTFRIATCANNALYGLIFPSADIKTKDASIVYCIIAIHKDEKSLFNPGALHATFKVPGGFLSISKSMRLDKKRCHRIVTSPGIFLTIATMLKGDNPTISLNDVLNFSIFASLNITKSMLSLTEPSRYMIMNSLAVSSHVREYISEKFSPYTKTLFSVHMVEKIKAGCLNAFKQREKIKTRDIYLTDIDITQKGIQDNRDLCSIWFDGNVTLKEYLNQIYIVFYLNPKALHEKHHVMIDLLKTVIEIELDQRENVPQPWSDVPKKQTVNLPILVHSLAKNLLLDTSFAHFLRSRIESRNNFRRTFATISTFTSSKSCLKTGNFHEFKIKQCQRLKKVNTSEAKKHRIANAMFVEEQDQHLEVEHANYELMRKAIPDYVDVLSTKVFDRLYELYKTGEIDDSPVIHQIFATMKSHTKFYFTYFNKGQKTAKDREIFVGEYEAKMCMYLVERIYKERSKVNPDEMISEPGDGKLRVLERKAEQEIRFMVEKMKAKNDEINKEIEDAKDNYVLNLGKIAALQAQKYKALKLEINADMSKWSAQDVFFKYFWSVCLDPILYPEEKEHILYFFCNYMQKELVIPDEVICNILDQRKAYPNDIISQITNGLTTNHFNVKRNWLQGNFNYMSSYAHSTAMSVFKDVIKRAADLLEAEVLIHSMVHSDDNQTSVTLVDNRICPKQFTAFVINTFEKICLTFGCQANMKKTYITNHIKEFVSLFNLYGEPFSIYGRFTLTSVGDCAYIGPYEDLASRISATQTGIKHGCPASQAWLSITIAQWMTYLTYNMLPGQQNDPWPILEIDRKQLPLELGGYISCPLSLIALAGLESGNIDFLIKLVNKYVDPRLQREPIQDQCTDIKNWDISRLSKVEIFKLKVLRYLVLDAEMDNTDIMGETSEMRGRSLLTPRKFTTAGSLRKLVSFEDFQAVQDTEQGVDVIVEYMLQNPALLVTKGETKDDYMNTVLYRYNSKKFKESLSIQNPTQLFLEQILFSHKPIVDYTGIAEKFSNLNDGTMLEDNPTIKGRMTFTDAFAMIKKDLSTLKITNEDLEIVLKFIILNDPLTVTAANAHILHVIGHSQPRLGSTACVMPEFRNLRMIKHSPALVLKCYSKNTLLLPGVQERDMERDLNHLKTFIETTRLEHKMQDRIKKNEDLKKSKDIYFEIKEVTRFYQTCYEYVKSTDYKVKVFILPAKCMTQTDFCAVLQGSLLEDKKWKLIQHLRPVTAGGHKGEVQPVVSMDFKLAREAVNLLCFFTDSFIDSRYRRDFLLKACVEMAYKDRPMVTLIEEIKKSKNRTSFLPFLYRIGELTQEDLDAYDAQKAGGRVTWNHWQSTRSLNMGKIDFQIDTHKSHLHIIGEDQQLVIAELKIPKLTANAITQAGYRLLNEKHGFRFETMNEVLVQPRKYYITYQMKSKKQYVYKIFDTATLLYERRNIKQYTGREANPIVAVCEVVPMEEEETPALSLSDIEMYNADNESVSILKTSFNESAKMRRANLSKMQYFETIGGSMLKIRFINVNALMKDTTLMSLNYDNLVNVDLARFSKLLDCDGDTESVEDGILCFSDDPMEQTTTEEIDAIPLFKVSYKIPTPARLTYKNAIRELLRREITRFMDAFTFVGPSFDSPENMGFICNICCIIQLLHTNEWSTIMLNCIHICMIYLEKDIRFHKFLLNRIFFEGLNPASGKLDYKKIKEFVISLKDREMAPWNEIFSKFKQKCVTLLDKEITRIEQNTNFENILALDESTDDQSGFLLFE

SEQ ID NO: 7 - DNA, 316 bp, artificial sequence
  synthetic polynucleotide (S segment target sequence (partial))
aaacgcagaactgggtagcactagcatttatccaggatggctgattctaagctcacatacgaggatacacaggatgttagtagaagtacttataacccagcagatgaatacgatacgtttgtgggtgtctacagagaatttctcacaattgataacattagaatcttcttcatcaacgctccaaaggccaaaactgcgatggctaaactcaagaccgagacagttgaagttacatttggaacactcgttgtcaagctggttaataaccatagaattggacaggctcagcgtgaggttgcggacgatgagctaactc

SEQ ID NO: 8 - DNA, 425 bp, artificial sequence
  synthetic polynucleotide (M segment target sequence)
acaggacaaatagcactaaaggtcttgttgggagactttaactacaagcagtatgctgcaaatgtagaggctgacatagaagcaaattgcgttgggtgtacaaattgtataaagggaataacatgtgaaataaaggtgaaaacagaaattgaagcatcatgtaaggtagagcccccatgcccctcttacacaagtagaattataataaaaccaggtagagacacccacacattattgatgaagtgtgacaaaaaaataacgactggtgaactagcaataaaaatatgtaatatgcaaatccaggctcatctttcaacaatagagagcaatgaccaactagaattgtcgactggggatcaatcaacatatatacatgaagaagacctaaggtgttcaacctggatctgcawwgtgagagacgaagg

SEQ ID NO: 9 - DNA, 457 bp, artificial sequence
  synthetic polynucleotide (L segment target sequence)
agaattggttatcccagatgaggttatctgcaatatcctagatcagaggaaagcataccctaatgacataattagtcagatcacaaatggcttgacaaccaaccatttcaatgtaaagagaaactggctacaaggcaacttcaattacatgtccagctatgctcacagtacagcaatgtctgtctttaaagatgtgataaagcgtgctgcagatttactagaagctgaagttctgattcattctatggttcactctgatgataaccagacctctgtaacattggtcgacaacaggatatgcccaaagcaattcacagcatttgtaatcaatacatttgaaaagatctgcctaacattcggctgtcaagctaatatgaaaaaaacctatatcaccaaccatataaaagaatttgtttcactattcaatttatatggagaaccattttcaatttatggc

SEQ ID NO: 10 - DNA, 20 bp, artificial sequence
  synthetic oligonucleotide (BunyaCladeS_Fw1)
aaacgcagaactgggtagca

SEQ ID NO: 11 - DNA, 20 bp, artificial sequence
  synthetic oligonucleotide (BunyaCladeS_Rv1)
gagttagctcatcgtccgca

SEQ ID NO: 12 - DNA, 23 bp, artificial sequence
  synthetic oligonucleotide (BunyaCladeM_Fw1)
acaggrcaaatagcactaaaggt

SEQ ID NO: 13 - DNA, 21 bp, artificial sequence
  synthetic oligonucleotide (BunyaCladeM_Rv1)
ccttcrtctctcactttgcag

SEQ ID NO: 14 - DNA, 24 bp, artificial sequence
  synthetic oligonucleotide (BunyaCladeL_Fw1)
agaattggttatcccagatgaggt

SEQ ID NO: 15 - DNA, 25 bp, synthetic oligonucleotide (BunyaCladeL_Rv1)
gccataaattgaaaatggttctcca

SEQ ID NO: 16 - DNA, 23 bp, artificial sequence
  synthetic oligonucleotide (BunyaUmbreM_Fw1)
ggatagtctcagattggaccaca

SEQ ID NO: 17 - DNA, 23 bp, artificial sequence
  synthetic oligonucleotide (BunyaUmbreM_Rv1)
tctgtgggttttcattgcatctg

SEQ ID NO: 18 - DNA, 22 bp, artificial sequence
  synthetic oligonucleotide (BunyaUmbreM_Fw2)
gcttaccaccctttcacaaagt

SEQ ID NO: 19 - DNA, 20 bp, artificial sequence
  synthetic oligonucleotide (BunyaUmbreM_Rv2)
gctgcggcagtcagcattat

SEQ ID NO: 20 - DNA, 22 bp, artificial sequence
  synthetic oligonucleotide (BunyaUmbreM_Fw3)
acgaaatcattgctctgccaac

SEQ ID NO: 21 - DNA, 20 bp, artificial sequence
  synthetic oligonucleotide (BunyaUmbreM_Rv3)
tgttgtgcttggctgcattt

SEQ ID NO: 22 - DNA, 22 bp, artificial sequence
  synthetic oligonucleotide (BunyaUmbreM_Fw4)
aaggaatctgagctaggacaag

SEQ ID NO: 23 - DNA, 23 bp, artificial sequence
  synthetic oligonucleotide (BunyaUmbreM_Rv4)
atctgttgttagcacacaatgtt

SEQ ID NO: 24 - DNA, 20 bp, artificial sequence
  synthetic oligonucleotide (BunyaUmbreM_Fw5)
ttgcaaagtgctcgcgaatg

SEQ ID NO: 25 - DNA, 20 bp, artificial sequence
  synthetic oligonucleotide (BunyaUmbreM_Rv5)
agccccaattgctggttctt

SEQ ID NO: 26 - DNA, 19 bp, artificial sequence
  synthetic oligonucleotide (BunyaUmbreM_Fw6)
gagcactgcacagggacat

SEQ ID NO: 27 - DNA, 20 bp, artificial sequence
  syntehtic oligonucleotide (BunyaUmbreM_Rv6)
cttgtgtaagaggggcatgg

SEQ ID NO: 28 - DNA, 19 bp, artificial sequence
  synthetic oligonucleotide (BunyaUmbreM5_Fw)
gtttgagattaccatcaag

SEQ ID NO: 29 - DNA, 23 bp, artificial sequence
  synthetic oligonucleotide (BunyaUmbreM5_Rv)
tgtggtccaatctgagactatcc

SEQ ID NO: 30 - DNA, 21 bp, artificial sequence
  synthetic oligonucleotide (BunyaUmbreM3_Fw)
ctgcaaagtgagagaygaagg

SEQ ID NO: 31 - DNA, 17 bp, artificial sequence
  synthetic oligonucleotide (BunyaUmbreM3_Rv)
catgactataccattga

SEQ ID NO: 32 - DNA, 22 bp, artificial sequence
  synthetic oligonucleotide (BunyaUmbreL3_Fw)
tcctgcatctgggaaattggat

SEQ ID NO: 33 - DNA, 24 bp, artificial sequence
  synthetic oligonucleotide (BunyaUmbreL3_Rv)
ctagagagaatagatgaactcttg

SEQ ID NO: 34 - DNA, 20 bp, artificial sequence
  synthetic oligonucleotide (BunyaUmbreL_Fw1)
acaggaacgatgttcggcta

SEQ ID NO: 35 - DNA, 21 bp, artificial sequence
  synthetic oligonucleotide (BunyaUmbreL_Rv1)
tctttgaatatcggatgccca

SEQ ID NO: 36 - DNA, 20 bp, artificial sequence
  synthetic oligonucleotide ( BunyaUmbreL_Fw1bis)
gttgcgagagcaaatgagcc

SEQ ID NO: 37 - DNA, 22 bp, artificial sequence
  artificial sequence (BunyaUmbreL_Rv1bis)
ttctttgaatatcggatgccca

SEQ ID NO: 38 - DNA, 23 bp, artificial sequence
  synthetic oligonucleotide (BunyaUmbreL_Fw2)
aagaacaaagggaagtgtcctca

SEQ ID NO: 39 - DNA, 23 bp, artificial sequence
  synthetic oligonucleotide (BunyaUmbreL_Rv2)
tctgtttcagtgtcatctaagcc

SEQ ID NO: 40 - DNA, 21 bp, artificial sequence
  synthetic oligonucleotide (BunyaUmbreL_Fw3)
ctggcaggtcgtcactcaata

SEQ ID NO: 41 - DNA, 22 bp, artificial sequence
  synthetic oligonucleotide (BunyaUmbreL_Rv3)
aatgcatttagacagcctgctt

SEQ ID NO: 42 - DNA, 25 bp, artificial sequence
  synthtetic oligonucleotide (BunyaUmbreL_Fw4)
tggtttgatggtaatgtcactttga

SEQ ID NO: 43 - DNA, 21 bp, artificial sequence
  synthetic oligonucleotide (BunyaUmbreL_Rv4)
tcgtctggattgactttcgat

SEQ ID NO: 44 - DNA, 20 bp, artificial sequence
  synthetic oligonucleotide (BunyaUmbreL_Fw5)
tgtaggggaatacgaggcca

SEQ ID NO: 45 - DNA, 22 bp, artificial sequence
  synthetic oligonucleotide (BunyaUmbreL_Rv5)
agggtatgctttcctctgatct

SEQ ID NO: 46 - DNA, 20 bp, artificial sequence
  synthetic oligonucleotide (BunyaUmbreL_Fw6)
ctgcctaacattcggctgtc

SEQ ID NO: 47 - DNA, 20 bp, artificial sequence
  synthetic oligonucleotide (BunyaUmbreL_Rv6)
tcttgcaccgcttggaaatc

SEQ ID NO: 48 - DNA, 22 bp, artificial sequence
  synthetic oligonucleotide (BunyaUmbreL_Fw6bis)
actgggacatttcaaggcttag

SEQ ID NO: 49 - DNA, 22 bp, artificial sequence
  synthetic oligonucleotide (BunyaUmbreL_Rv6bis)
gagaacttttctgcgatacctg

SEQ ID NO: 50 - DNA, 21 bp, artificial sequence
  synthetic oligonucleotide (BunyaUmbreL_Fw7)
actgatcaaggtgtggatgtt

SEQ ID NO: 51 - DNA, 20 bp, artificial sequence
  synthetic oligonucleotide (BunyaUmbreL_Rv7)
cgggcagcaacaaagtgttt

SEQ ID NO: 52 - DNA, 25 bp, artificial sequence
  synthetic oligonucleotide (BunyaUmbreL_Fw8)
gagcataaaatgcaagataggatca

SEQ ID NO: 53 - DNA, 20 bp, artificial sequence
  synthetic oligonucleotide (BunyaUmbreL_Rv8)
tcaaaccgaaacccatgctt

SEQ ID NO: 54 - DNA, 20 bp, artificial sequence
  synthetic oligonucleotide (BunyaUmbreL_Fw9)
aagcatgggtttcggtttga

SEQ ID NO: 55 - DNA, 21 bp, artificial sequence
  synthetic oligonucleotide (BunyaUmbreL_Rv9)
agccaggtcgacatttaccaa

SEQ ID NO: 56 - DNA, 22 bp, artificial sequence
  synthetic oligonucleotide (BunyaUmbreL_Fw10)
ttggactgtgacggtgatacag

SEQ ID NO: 57 - DNA, 22 bp, artificial sequence
  synthetic oligonucleotide (BunyaUmbreL_Rv10)
atccaatttcccagatgcagga

SEQ ID NO: 58 - protein, 285 aa, Moissiacense virus (Umbre orthobunyavirus strain Moissiacense)
QATIRCFSGGSKIMEKTSNVSLSELCLKDDVSQLKIIVDHTKNDSGLFSTASVWRKWIVSDWTTCNPKKMALGTISVIDIDKNFILKSSSYICNKECTITVDKERAQVLLQSDGLNHFEVSGTTLSSGWFKSTATVTLDQTCEHVKVSCGQKSMQFHACFKNHMSCIRFLHRSIMPASFAVSICQNIELILMTTFTLIIFLLLSILTKTYICYILLPIFIPFAYAYGFVYDKTCKKCSLCGLAYHPFTKCGIHCVCGCRFENSDAMKTHREKGKCPGFKSMRIAR

SEQ ID NO: 59 - protein, 174 aa, Moissiacense virus (Umbre orthobunyavirus strain Moissiacense)
VLCKAKGSAFALSVLLATLALGFLTPVQGLVLDKTQINYTEDQLPESFQTMQSTISIFKFATVMNAGWTYCMFLVTLALYIIHKKYAHRLLSYYVIHCRECDMLHDKSGLKYNGDFTNKCGFCTCGQVEDAMGLTVHQIRNHCSANYRTKMVLNWMIVLLLATLIKDSIMLTAA

SEQ ID NO: 60 - protein, 989 aa, Moissiacense virus (Umbre orthobunyavirus strain Moissiacense)
AGTEFETCIKKVEMTPECTGPFMEVGICDHQQKSLRYHEIANMLLGKGTISKLDVDIIDALPDRIAGDLQIIQSSSDFHHQQMLEYVFLLRHCDYYSSFVSDNSYSQILWQTAAKLNETNLCKHENSKKSCKCLKSNANCGESEDINIAAQAYYKNKESELGQDLTTIMYILKKMIPGSGYSYLLNAAKHNKLELFKAYMTNISSKYSNNKKLKDFMAIINAILANLSALSHSSEESISQYKQIDFSSLVGETTDMLEANFNQTISTDKIICENPKVMICISPRTKVSSGELYVCQRSGKYYIIDTGKFKLYKLIDADNLYCAADAQCRYEFRILTTGEMQATFKDNCKASVHVNTPGYQNEAITHCKVLANGKCKYNNQTSIDITLCANNRYYPEAKGRIFGVDPEDLCFDKTCTKQQTPYNEELISMCVWENPTLRPIKPRTEVSMTFQEYKDQLLKKINTDLVLHKFVRTQNLPYFIPQFKYITIQGTSTTDGITSSFIFFEIPALTGASAGYKVINSEGQELMDMVVYIKTSKTSAKYKRVYYTGPTIAINTKHQEHCTGTCPERIEHDEGWATFSKERTSNWGCEEFGCLAVETGCLFGSCQDVIRRELDVFSKLEEDKILTELCITLSHDTYCVTIDSTTPTINDYFEIQYKTVDVQTLPKMIGVTHHKLLRGQINELGSFGKFCGNIQVVGNQTYGQAAVKFDYICHAAQRKDVVIRKCLENNYQSCKLLTHDTDLILEESKTSVEVINNKRITGQIALKVLLGDFNYKQYAANVEADIEANCVGCTNCIKGITCEIKVKTEIEASCKVEPPCPSYTSRIIIKPGRDTHTLLMKCDKKITTGELAIKICNMQIQAHLSTIESNDQLELSTGDQSTYIHEEDLRCSTWICKVRDEGISFIFKPLTDWLGSFTKPILIAGCMIIVAIILIYILMPMCARLRDLLKKNEYEYLQDTKVIVKPKGTASSIGLRSKKINIQSSKAVD

SEQ ID NO: 61 - protein, 920 aa, artificial sequence
  synthetic polypeptide (Gc protein extracellular domain)
  VARIANT (897)..(897): Xaa is Isoleucine or Lysine
AGTEFETCIKKVEMTPECTGPFMEVGICDHQQKSLRYHEIANMLLGKGTISKLDVDIIDALPDRIAGDLQIIQSSSDFHHQQMLEYVFLLRHCDYYSSFVSDNSYSQILWQTAAKLNETNLCKHENSKKSCKCLKSNANCGESEDINIAAQAYYKNKESELGQDLTTIMYILKKMIPGSGYSYLLNAAKHNKLELFKAYMTNISSKYSNNKKLKDFMAIINAILANLSALSHSSEESISQYKQIDFSSLVGETTDMLEANFNQTISTDKIICENPKVMICISPRTKVSSGELYVCQRSGKYYIIDTGKFKLYKLIDADNLYCAADAQCRYEFRILTTGEMQATFKDNCKASVHVNTPGYQNEAITHCKVLANGKCKYNNQTSIDITLCANNRYYPEAKGRIFGVDPEDLCFDKTCTKQQTPYNEELISMCVWENPTLRPIKPRTEVSMTFQEYKDQLLKKINTDLVLHKFVRTQNLPYFIPQFKYITIQGTSTTDGITSSFIFFEIPALTGASAGYKVINSEGQELMDMVVYIKTSKTSAKYKRVYYTGPTIAINTKHQEHCTGTCPERIEHDEGWATFSKERTSNWGCEEFGCLAVETGCLFGSCQDVIRRELDVFSKLEEDKILTELCITLSHDTYCVTIDSTTPTINDYFEIQYKTVDVQTLPKMIGVTHHKLLRGQINELGSFGKFCGNIQVVGNQTYGQAAVKFDYICHAAQRKDVVIRKCLENNYQSCKLLTHDTDLILEESKTSVEVINNKRITGQIALKVLLGDFNYKQYAANVEADIEANCVGCTNCIKGITCEIKVKTEIEASCKVEPPCPSYTSRIIIKPGRDTHTLLMKCDKKITTGELAIKICNMQIQAHLSTIESNDQLELSTGDQSTYIHEEDLRCSTWICXVRDEGISFIFKPLTDWLGSFTKP

SEQ ID NO: 62 - protein, 261 aa, artificial sequence
  synthetic polypeptide (Gc protein N-terminal alpha helix region)
LRYHEIANMLLGKGTISKLDVDIIDALPDRIAGDLQIIQSSSDFHHQQMLEYVFLLRHCDYYSSFVSDNSYSQILWQTAAKLNETNLCKHENSKKSCKCLKSNANCGESEDINIAAQAYYKNKESELGQDLTTIMYILKKMIPGSGYSYLLNAAKHNKLELFKAYMTNISSKYSNNKKLKDFMAIINAILANLSALSHSSEESISQYKQIDFSSLVGETTDMLEANFNQTISTDKIICENPKVMICISPRTKVSSGELYVC

SEQ ID NO: 63 - protein, 431 aa, artificial sequence
  synthetic polypeptide (Gc protein N-terminal domain)
GTEFETCIKKVEMTPECTGPFMEVGICDHQQKSLRYHEIANMLLGKGTISKLDVDIIDALPDRIAGDLQIIQSSSDFHHQQMLEYVFLLRHCDYYSSFVSDNSYSQILWQTAAKLNETNLCKHENSKKSCKCLKSNANCGESEDINIAAQAYYKNKESELGQDLTTIMYILKKMIPGSGYSYLLNAAKHNKLELFKAYMTNISSKYSNNKKLKDFMAIINAILANLSALSHSSEESISQYKQIDFSSLVGETTDMLEANFNQTISTDKIICENPKVMICISPRTKVSSGELYVCQRSGKYYIIDTGKFKLYKLIDADNLYCAADAQCRYEFRILTTGEMQATFKDNCKASVHVNTPGYQNEAITHCKVLANGKCKYNNQTSIDITLCANNRYYPEAKGRIFGVDPEDLCFDKTCTKQQTPYNEELISMCVW

SEQ ID NO: 64 - protein, 254 aa, artificial sequence
  synthetic polypeptide (fragment of Gc protein N-terminal domain)
GTEFETCIKKVEMTPECTGPFMEVGICDHQQKSLRYHEIANMLLGKGTISKLDVDIIDALPDRIAGDLQIIQSSSDFHHQQMLEYVFLLRHCDYYSSFVSDNSYSQILWQTAAKLNETNLCKHENSKKSCKCLKSNANCGESEDINIAAQAYYKNKESELGQDLTTIMYILKKMIPGSGYSYLLNAAKHNKLELFKAYMTNISSKYSNNKKLKDFMAIINAILANLSALSHSSEESISQYKQIDFSSLVGETTD

SEQ ID NO: 65 - DNA, 2760 bp, artificial sequence
  synthetic polynucleotide coding for Gc protein extracellular domain
gcagggacagaatttgaaacatgcatcaagaaagtagaaatgacaccggaatgcacaggacctttcatggaagttggaatctgtgatcaccagcagaagagcctaagataccatgagatagctaatatgttattgggtaaagggacaatctcaaaattagatgtggatattatagatgcattgcctgacaggatagctggagacctccagataatacagtcaagcagtgatttccaccatcaacagatgctggaatatgtgtttctattgcgtcattgtgattattactcaagttttgtttcggataacagctactcacaaatcttgtggcaaacagcagcaaagttaaatgaaaccaacctttgcaaacatgagaattcaaagaaatcctgcaagtgcttaaaatcaaatgcaaattgtggagagtcagaagacatcaacatagcagcacaggcatactacaaaaataaggaatctgagctaggacaagatctaacaaccataatgtacatactcaaaaaaatgattccaggatcaggttatagttatctgctaaatgcagccaagcacaacaaattagaattgttcaaagcttacatgactaatatttcctcaaaatattcaaataacaaaaaattaaaagatttcatggcgataataaatgctatactagcaaatctgtcagctctctcacatagtagtgaagaatcaatctcacaatacaaacagattgatttttcttccctagtaggcgaaacaacagacatgctcgaagcaaattttaatcaaacgatcagtacagacaagataatttgtgaaaatcctaaagtaatgatttgcatttcacccaggacaaaagtttcatccggtgaattgtatgtctgccaaagatcaggaaagtactacataatagataccggcaaattcaagctatataaattaattgacgcagacaatttgtactgtgcagcagatgctcagtgtaggtatgaatttagaattttaaccacaggggaaatgcaggcaacttttaaagataattgcaaagcatcagtacatgttaacaccccaggataccaaaatgaagctataactcattgcaaagtgctcgcgaatggtaaatgtaagtataataatcaaacttcaatagatataacattgtgtgctaacaacagatattatcccgaagcaaaaggcaggatctttggagttgatccagaagatctatgctttgataagacatgtactaaacaacagactccatacaacgaagaactaatcagtatgtgtgtttgggaaaatccgacacttaggccaatcaaacccagaactgaggtttctatgactttccaagagtacaaagatcagttattaaagaaaatcaacacagacctggtgctgcacaaatttgttagaacacaaaacttaccttatttcataccgcaattcaagtatataactatacaaggaacgtcaacaacagacgggattacttccagttttatattctttgaaattcctgcattgacaggagcatctgctggatacaaagttataaatagcgaaggccaagaattgatggacatggtagtttatatcaaaacatcaaagactagcgcaaagtacaagcgcgtgtattatacaggccccactatagctataaatacaaaacatcaagagcactgcacagggacatgtcctgaaagaatagaacatgatgaaggttgggcaacattttcgaaagaaagaaccagcaattggggctgtgaagaatttggttgtctagctgttgagactggttgtttatttgggtcatgccaggatgtaattagaagagaacttgatgttttttcaaagttggaggaagataaaatattgactgaactctgtataacattaagccatgacacttactgcgtgacaatcgattctacaacaccaacaatcaatgattactttgaaatccaatacaaaacagtagatgtacaaacattgccaaagatgataggagtcactcatcataagctattgcgagggcagataaacgaattaggatcatttggcaaattttgtggcaacatacaagtagttggtaatcaaacatatgggcaggctgcagtaaagtttgattacatttgccatgctgcacaaagaaaagatgtagttataagaaagtgcttagaaaataattaccaaagttgtaagctactgacacatgacacagacttgatacttgaagaaagtaagaccagtgttgaagtcataaacaataaaaggattacaggacaaatagcactaaaggtcttgttgggagactttaactacaagcagtatgctgcaaatgtagaggctgacatagaagcaaattgcgttgggtgtacaaattgtataaagggaataacatgtgaaataaaggtgaaaacagaaattgaagcatcatgtaaggtagagcccccatgcccctcttacacaagtagaattataataaaaccaggtagagacacccacacattattgatgaagtgtgacaaaaaaataacgactggtgaactagcaataaaaatatgtaatatgcaaatccaggctcatctttcaacaatagagagcaatgaccaactagaattgtcgactggggatcaatcaacatatatacatgaagaagacctaaggtgttcaacctggatctgcawwgtgagagacgaagggataagcttcatctttaagccattaacagactggcttggaagcttcacaaagccg

SEQ ID NO: 66 - DNA, 783 bp, artificial sequence
  synthetic polynucleotide coding fo Gc protein N-terminal alpha-helix  region
ctaagataccatgagatagctaatatgttattgggtaaagggacaatctcaaaattagatgtggatattatagatgcattgcctgacaggatagctggagacctccagataatacagtcaagcagtgatttccaccatcaacagatgctggaatatgtgtttctattgcgtcattgtgattattactcaagttttgtttcggataacagctactcacaaatcttgtggcaaacagcagcaaagttaaatgaaaccaacctttgcaaacatgagaattcaaagaaatcctgcaagtgcttaaaatcaaatgcaaattgtggagagtcagaagacatcaacatagcagcacaggcatactacaaaaataaggaatctgagctaggacaagatctaacaaccataatgtacatactcaaaaaaatgattccaggatcaggttatagttatctgctaaatgcagccaagcacaacaaattagaattgttcaaagcttacatgactaatatttcctcaaaatattcaaataacaaaaaattaaaagatttcatggcgataataaatgctatactagcaaatctgtcagctctctcacatagtagtgaagaatcaatctcacaatacaaacagattgatttttcttccctagtaggcgaaacaacagacatgctcgaagcaaattttaatcaaacgatcagtacagacaagataatttgtgaaaatcctaaagtaatgatttgcatttcacccaggacaaaagtttcatccggtgaattgtatgtctgc

SEQ ID NO: 67 - DNA, 1293 bp, artificial sequence
  synthetic polynucleotide coding for Gc prootein N-terminal domain
gggacagaatttgaaacatgcatcaagaaagtagaaatgacaccggaatgcacaggacctttcatggaagttggaatctgtgatcaccagcagaagagcctaagataccatgagatagctaatatgttattgggtaaagggacaatctcaaaattagatgtggatattatagatgcattgcctgacaggatagctggagacctccagataatacagtcaagcagtgatttccaccatcaacagatgctggaatatgtgtttctattgcgtcattgtgattattactcaagttttgtttcggataacagctactcacaaatcttgtggcaaacagcagcaaagttaaatgaaaccaacctttgcaaacatgagaattcaaagaaatcctgcaagtgcttaaaatcaaatgcaaattgtggagagtcagaagacatcaacatagcagcacaggcatactacaaaaataaggaatctgagctaggacaagatctaacaaccataatgtacatactcaaaaaaatgattccaggatcaggttatagttatctgctaaatgcagccaagcacaacaaattagaattgttcaaagcttacatgactaatatttcctcaaaatattcaaataacaaaaaattaaaagatttcatggcgataataaatgctatactagcaaatctgtcagctctctcacatagtagtgaagaatcaatctcacaatacaaacagattgatttttcttccctagtaggcgaaacaacagacatgctcgaagcaaattttaatcaaacgatcagtacagacaagataatttgtgaaaatcctaaagtaatgatttgcatttcacccaggacaaaagtttcatccggtgaattgtatgtctgccaaagatcaggaaagtactacataatagataccggcaaattcaagctatataaattaattgacgcagacaatttgtactgtgcagcagatgctcagtgtaggtatgaatttagaattttaaccacaggggaaatgcaggcaacttttaaagataattgcaaagcatcagtacatgttaacaccccaggataccaaaatgaagctataactcattgcaaagtgctcgcgaatggtaaatgtaagtataataatcaaacttcaatagatataacattgtgtgctaacaacagatattatcccgaagcaaaaggcaggatctttggagttgatccagaagatctatgctttgataagacatgtactaaacaacagactccatacaacgaagaactaatcagtatgtgtgtttgg

SEQ ID NO: 68 - DNA, 762 bp, artificial sequence
  synthetic polynucleotide coding for fragment of Gc protein N-terminal domain
gggacagaatttgaaacatgcatcaagaaagtagaaatgacaccggaatgcacaggacctttcatggaagttggaatctgtgatcaccagcagaagagcctaagataccatgagatagctaatatgttattgggtaaagggacaatctcaaaattagatgtggatattatagatgcattgcctgacaggatagctggagacctccagataatacagtcaagcagtgatttccaccatcaacagatgctggaatatgtgtttctattgcgtcattgtgattattactcaagttttgtttcggataacagctactcacaaatcttgtggcaaacagcagcaaagttaaatgaaaccaacctttgcaaacatgagaattcaaagaaatcctgcaagtgcttaaaatcaaatgcaaattgtggagagtcagaagacatcaacatagcagcacaggcatactacaaaaataaggaatctgagctaggacaagatctaacaaccataatgtacatactcaaaaaaatgattccaggatcaggttatagttatctgctaaatgcagccaagcacaacaaattagaattgttcaaagcttacatgactaatatttcctcaaaatattcaaataacaaaaaattaaaagatttcatggcgataataaatgctatactagcaaatctgtcagctctctcacatagtagtgaagaatcaatctcacaatacaaacagattgatttttcttccctagtaggcgaaacaacagac

SEQ ID NO: 69 - DNA, 19 bp, artificial sequence
  synthetic oligonucleotide (Koongol virus L segment forward primer)
gacccaatactgtaaacag

SEQ ID NO: 70 - DNA, 18 bp, artificial sequence
  synthetic oligonucleotide (Koongol virus L segment reverse primer)
cgtcagaatgcaccattg

SEQ ID NO: 71 - DNA, 240 bp, Moissiacense virus (Umbre orthobunyavirus strain Moissiacense)
  CDS (1)..(240)
atgttagtagaagtacttataacccagcagatgaatacgatacgtttgtgggtgtctacagagaatttctcacaattgataacattagaatcttcttcatcaacgctccaaaggccaaaactgcgatggctaaactcaagaccgagacagttgaagttacatttggaacactcgttgtcaagctggttaataaccatagaattggacaggctcagcgtgaggttgcggacgatgagctaa

SEQ ID NO: 72 - protein, 79 aa, Moissiacense virus (Umbre orthobunyavirus strain Moissiacense)
MLVEVLITQQMNTIRLWVSTENFSQLITLESSSSTLQRPKLRWLNSRPRQLKLHLEHSLSSWLITIELDRLSVRLRTMS

SEQ ID NO: 73 - DNA, 714 bp, moissiacense virus (Umbre orthobunyavirus strain Moissiacense)
atggctgattctaagctcacatacgaggatacacaggatgttagtagaagtacttataacccagcagatgaatacgatacgtttgtgggtgtctacagagaatttctcacaattgataacattagaatcttcttcatcaacgctccaaaggccaaaactgcgatggctaaactcaagaccgagacagttgaagttacatttggaacactcgttgtcaagctggttaataaccatagaattggacaggctcagcgtgaggttgcggacgatgagctaactcttcaccgactttctggctacattgcaaagtacactcttcacctatacaaaaatgcaaaaaaagcaggagagagagaagcaataataaccaagatcgttaatccaatttctgccaaaatgggcttccaatggagtgttgggccggaaatttatctctcaacgctgccaggaaccgaaatgtttctagatacatttaaaatgttcccattggcattcatcttgttaagagttaaaagaggagagatcaaggtggaaatggcaaaaaaagcaatgcggcagaagtatggcgacaaagatgccagtgaatggctgcaggaggacattgagactgtaaaaggggcaataaaaacagttgaaaagctcaagccaacgctgacaggattggctgcttcaatgactgctttcctgcaacaacttggtatcaacactaagtaa

SEQ ID NO: 74 - RNA, 24 nt, artificial sequence
  Cal/Bwa group Fw primer (RNA equivalent)
gcaaauggauuugauccugaugca

SEQ ID NO: 75 - RNA, 25 nt, artificial sequence
  Cal/Bwa group RV primer (RNA equivalent)
uuguuccuguuugcuggaaaaugau

SEQ ID NO: 76 - RNA, 25 nt, artificial sequence
  Moissiacense virus genomic sequence
agaaguacuuauaacccagcagaug

SEQ ID NO: 77 - RNA, 25 nt, artificial sequence
  Moissiacense virus genomic sequence
cgcugagccuguccaauucuauggu

SEQ ID NO: 78 - RNA, 26 nt, artificial sequence
  Bunyamwera group Fw primer (RNA equivalent)
cugcuaacaccagcaguacuuuugac

SEQ ID NO: 79 - RNA, 28 nt, artificial sequence
  Bunyamwera group Rv primer (RNA equivalent)
uggaggguaagaccaucgucaggaacug

SEQ ID NO: 80 - RNA, 26 nt, artificial sequence
  Moissiacense virus genomic sequence
aggauguuaguagaaguacuuauaac

SEQ ID NO: 81 - RNA, 28 nt, artificial sequence
  Moissiacense virus sequence
ugaagaguuagcucaucguccgcaaccu

SEQ ID NO: 82 - RNA, 29 nt, artificial sequence
  Wyeomyia Fw primer (RNA equivalent)
augucugaaauuguauuugaugauauugg

SEQ ID NO: 83 - RNA, 21 nt, artificial sequence
  Wyeomyia Rv primer (RNA equivalent)
uauuucgauuccccggaaagu

SEQ ID NO: 84 - RNA, 29 nt, artificial sequence
  Moissiacense virus genomic sequence
gauucuaagcucacauacgaggauacaca

SEQ ID NO: 85 - RNA, 21 nt, artificial sequence
  Moissiacense virus genomic sequence
gcugagccuguccaauucuau

SEQ ID NO: 86 - RNA, 22 nt, artificial sequence
  Oropouche Fw primer (RNA equivalent)
ggcccaugguugaccuuacuuu

SEQ ID NO: 87 - RNA, 21 nt, artificial sequence
  Oropouche Rv primer (RNA equivalent)
accaaagggaagaaagugaau

SEQ ID NO: 88 - RNA, 22 nt, artificial sequence
  Moissiacense virus genomic sequence
ccgagacaguugaaguuacauu

SEQ ID NO: 89 - RNA, 21 nt, artificial sequence
  Moissiacense virus genomic sequence
gccaaugggaacauuuuaaau

SEQ ID NO: 90 - DNA, 714 bp, Umbre orthobunyavirus strain Marna
atggctgattctaaactcacatacgaggatacgcaggatgttagtagaagtacttataacccagcagatgaatacgatacgtttgtgggtgtctacagagaatttctcacaattgataacattagaatcttcttcatcaacgctccaaaggccaaagctgcgatggctaaactcaagaccgagacagttgaagttacgtttggaacactcgtcgtcaagctggttaataaccatagaattggacaggctcagcgtgaggttgcggacgatgagctaactcttcaccggctttctggctacattgcgaagtacactcttcacctatacaagaatgcaaaaaaagcaggagagagagaagcaataacaaccaaaatagttaatccaatttctgccaaaatgggcttccaatggagcgttgggccagaaatttacctttcaacactgccaggaactgaaatgtttctagatacatttaaaatgttcccattggcattcatcttggtgagagttaagagaggagaaatcaaggtagagatggcgaaaaaagcaatgcggcagaaatatggcgacaaagatgccagtgaatggctgcaggaggacattgagactgtgaaaggggcaataaaaacagttgaaaagctcaagccaacgctgacaggattggctgcttcaatgaccgctttcctgcaacaacttggtatcaacactaagtaa

SEQ ID NO: 91 - DNA, 4389 bp, Umbre orthobunyavirus strain Marna
atggtgatctttgcattgttgttgatattattggttgggttcagcaatcaagcgactattcgatgcttctctggcggctccaaaattatggaaaaaacatcgaatgtctcattgagtgagttatgcttgaaggatgatgtaagccagctaaaaattatagttgaccacactaaaaatgactcaggattgttttcaactgccagcgtctggagaaaatggatagtttcagactggaccacatgcaaccctaaaaaaatggccttgggaactatatctgtcatagacatcgataagaactttatcttaaaaagctccagctacatatgcaataaagagtgcacgataacagtagataaagaaagggcccaagttttgctacagtcggatggattaaaccattttgaggtttctggaaccactttaagttctggatggtttaaactgacagccactgttaccttagaccaaacttgcgagcatgttaaagtgtcttgtggtcaaaaatcaatgcaattccatgcctgtttcaagaatcatatgtcatgcattagattcttgcatagaagtataatgccagcaagctttgcagtttccatctgccaaaatatagagttgatattaatgacaacatttacactgattatatttttgctattgagcattttgaccaaaacatacatatgctacattttgctacccatatttatacccttcgcgtacgcatacggattcatttatgataagacatgcaagaagtgctcattgtgtgggttggcttatcacccttttacaaagtgtgggacacactgcgtctgtggatgtagatttgaaaattcagatgcaatgaaaacccacagagaaaaagggaaatgtccgggattcaagtcaatgagaactgctagggtactatgtaaggctaaaggttcagctttcactttatctgtactattggccacattagcattgggcttcttgacgcctgtgcaagggctagttttagatgagacccaaattagttacacagaagatcaattaccagaatcatttcaggtgatgcaatcaacaatatccatattcaaatttgcaacaattatgaatgcaggttggacttactgcatgttcctagttacattggctttatatatcatatacaagaagtatgcccacaggttattaagctattatgtgatacattgcaaggagtgtgatatgcttcatgacaaaagtgggcttaagtataatggtgattttactaacaaatgcgggttttgcacatgtgagcaagttgaagatgcaatggggctgactgtccatcaaatacgaaatcattgctctgccaattatagaactaagttggtgctgaactggatggttgtactattattagctactctaatcaagaatagcataatgttgactactgcagcagggacagaatttgaaacatgcatcaagaaagtagaaatgacacctgaatgcacaggacctttcatggaagttggaatctgtaatcaccaacaaaaaagcttaagataccacgagatagctaatatgttattgggtaaagggacaatctcaaaattagatgtggacattatagatgcattgcctgacaagatagctggagacctccaggtaatacaatcaagcagtgatttccatcatcagcagatgctggagtatgtgtttctattacgtcattgtgattactactcaagttttgtttcagataacagctactcgcaaattttatggcaaacagcagcaaaattaaatgaaatcaacctttgcaaacatgagagttcaaaaaagtcctgcaagtgcttaaaatcaaatgcaaattgtggagagtcagaagacatcaatacagcagcacaggcatattacaaaaataaagagtctgagctaggacaggatttaacaaccataatgtacatactcaaaaaaatgattccaggatcaggttatagttatctgctaaatgcaactaagcacaacaaattagaattgtttaaagcttacatgactaatatttcttcaaaatatccaaacaacaagaaattaaaagattttgtggcaataacaaatgctatactagcagatctatcagctctctcgcatagtagtgaagaatcaatcccagaatataagcagattgacttttcttccctagtaggtgaaacaacagacatgcttgaagcaaattttaatcaaacaatcagcacagacaagatagtttgcgaaaatcctaaagtaatgatttgcatttcaccaagagtttcatctggtgaattatatgtctgccaaaaattgggaaagtactacataatagatactggcaggtttaagttatataaattggttgatgcagacaatttgtactgtgcagcagatgctcagtgcaggtatgaatttagaattctaaccacaggagaaatgcaggcaacttttaaagataattgtaaagcatcaatacatactaacaccccaggatatcagaatgaagctataactcactgcaaggtgcttgcgaatgggaaatgtaaatatgacaatcaaactttaatagacgtaacattgtgtgctaacaacagatattatcccgaagcaaagggcaggatttttggagttgatccagaagatctatgctttgacaagacatgcaccaagctacaaactccatacaacgaagaactcatcagtatgtgtgtttgggaaaatccgacacttagaccaatcagacccagaactgagatttccatgactttccaagagtacaaagatcagttactaaaaaaaatcaacacagatctggtgctgcataaatttgttagaacacaaaacttgccttatttcataccgcaatttaagtacataactatacaaggaacgtcaacaacagatgggattacttccagttttatattctttgaaatccctgcactgacaggggcatctgctggatacaaagttataaatagtgaaggtcaagaactaatggacatggtagtttatgtcaaaacatcaaaaaccagcgcaaagtataagcgcatgtactatacaggccccactatagctataaatgcaaaacatcaagagcactgcacaggcacatgtcctgaaaggatagaacatgatgacggttgggcaacattttcgaaagaaagaaccagcaattgggggtgtgaagaatttggttgtctagctgttgagactggttgtttatttgggtcatgccaggatgtaattagaagagaactcgatgttttttcaaaattggaggaagataaaatattgactgaactctgtataacattaagtcatgacacttactgcgtgacaattgactctacaacaccaacaatcaatgattactttgaaattcaatataaaacagtagatgtacaaacattgccaaagatgataggggtcactcatcataagctattgcgagggcagataaacgaattagggtcatttggcaaattttgtggcgacatacaagtagttggtaatcaaacatatgggcaagctgcagtgaagtttgattacatctgtcatgctgcacagagaaaagatgtagttataagaaaatgcttagagaataattaccaaagttgtaagctactgacacatgacacagacttgatmcttgaagaaagtgagactagcgttgaagtcataaacaacaaaaggattacaggacaaatagcactaaaagtcttgttgggagactttaactacaagcagtatgctgcaaatgtggaagctgacatagaagcaaattgtgttggatgtacaaattgtataaaagggataacatgtgaaataaaggtgaaaacagaaattgaagcatcatgcaaagtagagcccccatgtccttcttacacgaatagaattataataaaaccaggtagagacacccacacattgttgatgaagtgtgacaaaaaaataatgactggtgaattagcaataaagatatgtaatatgcaaatccaagctcatctttcaacaatagaaagtaatgaccaactagaattgtcaactggggatcaatcaacatatatacatgaagaagacctaaggtgctcaacctggatctgcaaagtgagagatgaagggataagcttcatctttaagccattgacagattggcttggaagcttcacaaaaccaatacttatagctggctgcataataattgtcgcaattattttgatttatatattaatgcctatgtgtgctaagctcagagatttgttaaaaaagaacgagtatgaatatctacaagatacaaaagtgattgtaaagcccaaggctacagctagctcaatcggcttgagatcgaagaaaataaatatccaatcatctaaagcagttgattaa

SEQ ID NO: 92 - DNA, 6828 bp, Umbre orthobunyavirus strain Marna
atgttggatcaagaaaatgagcaagctttaaatagacttgcagctacagttgcaagagcaaatgagcctgccgaaggtaaagaagcatataatgctatactgagtagaaggcatgactactttgggcaagttttttgcgagactataggcataccatatagaaacgatgttcggctagaagatatcctacatgaatgcgaccaaacagttgacactctaacaaataaaataccaaacataactccagacaatttcgagtttagagacaatatcctaactattatagattataaagtggcagttagtgatgaaagtgctgactatactcgtgaaaagtatgaaaatgctgttgatgctataaagcatttggttgacttccctattagagtgtgtatagttaggatacatccatacactagacaagttacttactcagatgacaactttatgagacgatttgcccatgtggtataccctgttgattttacaagatacactcaattgactgaagaactcaaggaaaaatttgcagatagccctgagtttatggatatgatagcatatggcgatgtcacttttactgcaaactggtgtcaaaatggatgccctgagttgtacgagcatccaatatttaaagagtttttagagagcatgccattgaaataccagaaattgtttgaaaaatctttactaagctcttgctatacttctgagagatgggattccaatcttaaagaagtcaaggctgcaactaaagatgagtatgaagatttcatatctcgatctgcaaaacaactctatacaacatctcctgactattcagaacctagtcgagaggaaattctaaaagggtgggaagaaatgacagaaagagtgaaagaacaaagggaagtatcctcaaatattaatgaccaaaaaccaagtgctcacttcatatgggctgaaaacaatcacgaactgcctactgcaaattctgctaagatatgtgcaatttcaaaacttctacagtccattaatatagaaagctcttttgctgaagattttaaaagactaggcaaattattcgacttttctgaagatattcctggatatgagcgacattgcgaacaacttaaaaggcaggctagatcaaatccaggacaaataaaaaccaaaaaactagacccaaagaaaattgggaatgcattagttttatgggagcaacaatttttattatctgcagacgaaatgggaaaagagaataagctacacctacttaaagacttctttggcatagggaaacataagcaatttgcaagaaaaggcctagatgacaccgaaacagacaaaccaacaatcttagatttcaatgatacagaagtcaaaagatcagcagaattaatgatgcaaaaaacaaaactctacttatctggcaaatcatcactcaataaagagcatcctatagcatcagaatatcttaatgaaataaaaaagtgtaatgacgagacatataatgtccttaatgcgatctttcagacaaagtattggcaatgtatcacagacattagcatgctaatgaaaaatatgctatctgtgtcacagtataatagaaacaatactttcagaattgcaacatgtgctaataatgcactatatggacttatttttccatcagcagacattaaaacaaaggatgcaagcattgtatattgcattattgcaattcacaaagatgagaagtctttattcaatccaggagctctgcatgcaacttttaaagtgccaggtggctttttatctatatctaaatcaatgcggctcgacaagaagcgctgccatagaatagttactagtccaggcatattcttaacaattgccaccatgttgaaaggggacaatccaaccattagtctaaacgatgtcttaaattttagcatttttgcaagcttgaacataactaagagcatgctatcattaacagagccttctaggtatatgatcatgaactcgctagcagtctctagtcatgtacgagaatatatctctgagaaattttcaccatatactaaaactctctttagtgtccatatggttgagaaaataaaagcaggttgcctaaatgcattcaaacaaagagaaaaaatcaagactcgggacatatacttgacagacatagatataactcaaaaagggatacaagataacagagatctatgtagcatatggtttgatggtaatgtcactttgaaagaatatctgaatcagatttatattgtcttttatctgaatccgaaggcattgcatgaaaagcatcatgtaatgatagatctacttaaaacagtgatagaaatagaacttgatcaaagggagaatgtccctcaaccatggtctgatgtccctaaaaagcagactgtcaagttacccattcttgttcatagcctggcaaagaatctactcttggacacttcatttgcacatttcttaagatctagaattgaaagtcgcaataattttagacgcacgtttgcaacaatttcaacctttacaagtagtaagagttgcttaaaaacaggcaatttccatgaattcaagattaagcaatgtcaaaggctcaaaaaagtgaatgcgagtgaagcaaagaaacatagaatagcaaatgctatgtttgtcgaggaacaagatcaacatttggaggtggagcatgcaaactacgaattgatgaggaaggcaatcccggattatgtggatgtcttatcaaccaaggtatttgatagattgtatgagttatacaaaactggagaaatcgacgatagtcctgttatccaccagatttttgcgaccatgaaaagtcacactaaattctacttcacttattttaacaagggccaaaagacagcaaaagaccgagaaatattcgtaggggaatatgaggccaaaatgtgcatgtacctggtagaaagaatatataaagagagatcgaaagtcaatccagacgagatgatcagtgaaccaggagatgggaaactcagagtgttagagcgcaaagcagagcaagagataagattcatggttgaaaaaatgaaagcaaagaatgatgaaataaataaggaaatcgaggatgcaaaagacaattatgtcttaaatctagggaaaatagcagctttgcaagcacaaaaatacaaagctttaaaattggaaatcaatgcagacatgtcaaagtggagtgctcaggatgtattttttaaatacttttggtctatctgtcttgacccgattctctatcctgaagaaaaagaacacattttatattttttttgtaattatatgcaaaaagaattggttatcccagacgaagttatctgtaacatcctagaccagaggaaagcataccctaatgacataattagccagatcacaaatggattgacaactaaccatttcaatgtaaaaaggaactggctacaaggcaatttcaattacatgtccagctatgctcacagtacagcaatgtctgtctttaaagatgtgataaagcgtgctgcagatttactagaagctgaagttttgattcattctatggttcactctgatgataatcaaacctctgtaacattagttgacaataggatatgcccaaagcaattcacagcatttgtaatcaatacatttgaaaagatctgcctgacatttggctgtcaagccaatatgaaaaaaacctatatcaccaaccatataaaagaatttgtttcattatttaatttatatggggaaccattttcaatttacggcagattcacattaacatctgttggagactgtgcatacattggaccatatgaagacctcgcaagcagaatatcagcaacacagactgggataaagcatggatgcccagctagccaagcctggttatcaattgctatcgcccaatggatgacttatttgacatacaatatgttgccaggccaacaaaatgatccccagccaatattagaaatcgatagaaagcaattgccacttgaattgggtgggtacatttcttgtcctctatccttaatagctttagctggattggaatctggaaacattgatttcctgatcaaattagtaaacaaatatatcgaccccagacttcaacgtgaacctattcaagaccaatgcactgatataaagaactgggatatttcaaaacttagcaaagttgaaatatttaagctaaaagtgctgcgctatttagttttagatgcagagatggataatactgacattatgggagaaaccagtgagatgagaggaagatctctactaacacccagaaagttcacaacagctgggtctttgaggaaattagtatcttttgaagacttccaggcggtccaagattctgaacaaggtgtggattctatagttgagtacatgttgcaaaacccagcattacttgtgacaaagggagaaacaaaagacgactatatgaacactgtgctctatagatacaactcaaagaaatttaaagaatcattatctattcagaaccctactcagctcttcttggaacaaatcctattctcgcacaaacctattgttgattatacaggtatcgcagaaaaattctcaaatcttaatgatggaaccatgcttgaagataatccgacaataaaaggtagaatgaccttcacagatgctttcgcaatgattaagaaagatctatcaacactcagaatcactaatgaggatcttgaaattgttctaaaatttataattttgaatgaccctttaactgtgactgctgctaatgcccatatcttgcatgtaataggccattcacaacccaggcttgggtcaacagcttgtgttatgcctgaatttaggaatttgagaatgataaaacattcacctgcactagtcttgaagtgttatagtaaaaacactttgttgctgcctggggtgcaagaaagggacatggaaagagaccttaaccatctaaaaacatttattgagactacaagattagagcataaaatgcaagatagaattaagaaaaatgaagatctcaaaaaatcaaaggatatttacttcgaaatcaaagaggtaaccagattttatcaaacatgctatgaatatgtcaaaagtactgattataaggtaaaagtattcatattgccagccaaatgtatgactcaaacagatttttgtgctgtattacagggttcattattagaagataaaaagtggaaattaatacaacaccttagacctgttactgcaggtggccataaaggagaggttcaaccagtagtttccatggattttaaactagcacgagaggccgtgaatttgttatgttttttcactgattcattcatagactctagatataggagagactttcttctaaaagcatgcgtagaaatggcttataaagataggcctatggtcacattgatagaagaaataaagaagtcaaagaacagaacatctttcttaccattcttgtatagaattggtgagttaactcaagaagacctcgatgcatatgatgctcaaaaggctgggggaagagtaacctggaatcactggcagtccacaagaagtttgaacatgggaaagatagattttcaaatagatacacacaaaactcatctccatattattggtgaagatcaacaactggtgatagcagaactaaaaattcctaagttgacagcaaatgccatcactcaagcagggtatagacttttgaatgaaaagcatgggtttcggtttgaaacgatgaatgaagttttagtccagccaagaaaatattatataacataccagatgaaatctaaaaagcaatatgtctataaaatctttgacacagcgacgttgctatatgaaagaagaaatataaagcaatacacaggtcgagaagcaaatcccatagtagcagtctgtgaagttgttccaatggaggaggaggaaactcctgctttaagcctaagcgacatagaaatgtataatgctgacaacgaatcagttagtattttaaaaacatcatttaatgagagtgctaagatgagacgtgcaaacttgtccaaaatgcaatattttgagactattggaggatcaatgttgaaaattcgattcatcaatgttaatgcactaatgaaagacacaactctaatgtcccttaactatgacaatctggtaaatgttgatctagctagatttagcaagttattggactgtgacggtgacacagaaagtgttgaagatggcatattgtgcttttctgatgacccaatggaacaaaccacaacagaagagatcgatgcaattcctctctttaaagtaagctacaagatatcagcacctgccagattaacatacaagaatgccattagggaactgttaaggagggaaataacaaggtttatggatgcttttacctttgttggaccttcttttgattctccagaaaatatggggttcatatgcaatatatgttgtataatacaactcctccatacaaacgaatggtctatcataatgctaaactgtatccacatctgcatgatatatttggaaaaagacataaggttccataaatttctgctaaatagaatattttttgaggggttgaatcctgcatctggaaaattggattacaagaaaattaaagaatttgtaatcagcctgaaagatagggagatggctccttggaatgagatattttcaaaattcaagcaaaaatgtgtcacattgctagataaagaaataacaagaatagaacaaaacacaaactttgaaaacatactagctttagatgaaaacacagatgatcagtctgaattcctcttgtttgaatag

SEQ ID NO: 93 - protein, 237 aa, Umbre orthobunyavirus strain Marna
MADSKLTYEDTQDVSRSTYNPADEYDTFVGVYREFLTIDNIRIFFINAPKAKAAMAKLKTETVEVTFGTLVVKLVNNHRIGQAQREVADDELTLHRLSGYIAKYTLHLYKNAKKAGEREAITTKIVNPISAKMGFQWSVGPEIYLSTLPGTEMFLDTFKMFPLAFILVRVKRGEIKVEMAKKAMRQKYGDKDASEWLQEDIETVKGAIKTVEKLKPTLTGLAASMTAFLQQLGINTK

SEQ ID NO: 94 - protein, 90 aa, Umbre orthobunyavirus strain Marna
MILNSHTRIRRMLVEVLITQQMNTIRLWVSTENFSQLITLESSSSTLQRPKLRWLNSRPRQLKLRLEHSSSSWLITIELDRLSVRLRTMS

SEQ ID NO: 95 - protein, 1462 aa, Umbre orthobunyavirus strain Marna
MVIFALLLILLVGFSNQATIRCFSGGSKIMEKTSNVSLSELCLKDDVSQLKIIVDHTKNDSGLFSTASVWRKWIVSDWTTCNPKKMALGTISVIDIDKNFILKSSSYICNKECTITVDKERAQVLLQSDGLNHFEVSGTTLSSGWFKLTATVTLDQTCEHVKVSCGQKSMQFHACFKNHMSCIRFLHRSIMPASFAVSICQNIELILMTTFTLIIFLLLSILTKTYICYILLPIFIPFAYAYGFIYDKTCKKCSLCGLAYHPFTKCGTHCVCGCRFENSDAMKTHREKGKCPGFKSMRTARVLCKAKGSAFTLSVLLATLALGFLTPVQGLVLDETQISYTEDQLPESFQVMQSTISIFKFATIMNAGWTYCMFLVTLALYIIYKKYAHRLLSYYVIHCKECDMLHDKSGLKYNGDFTNKCGFCTCEQVEDAMGLTVHQIRNHCSANYRTKLVLNWMVVLLLATLIKNSIMLTTAAGTEFETCIKKVEMTPECTGPFMEVGICNHQQKSLRYHEIANMLLGKGTISKLDVDIIDALPDKIAGDLQVIQSSSDFHHQQMLEYVFLLRHCDYYSSFVSDNSYSQILWQTAAKLNEINLCKHESSKKSCKCLKSNANCGESEDINTAAQAYYKNKESELGQDLTTIMYILKKMIPGSGYSYLLNATKHNKLELFKAYMTNISSKYPNNKKLKDFVAITNAILADLSALSHSSEESIPEYKQIDFSSLVGETTDMLEANFNQTISTDKIVCENPKVMICISPRVSSGELYVCQKLGKYYIIDTGRFKLYKLVDADNLYCAADAQCRYEFRILTTGEMQATFKDNCKASIHTNTPGYQNEAITHCKVLANGKCKYDNQTLIDVTLCANNRYYPEAKGRIFGVDPEDLCFDKTCTKLQTPYNEELISMCVWENPTLRPIRPRTEISMTFQEYKDQLLKKINTDLVLHKFVRTQNLPYFIPQFKYITIQGTSTTDGITSSFIFFEIPALTGASAGYKVINSEGQELMDMVVYVKTSKTSAKYKRMYYTGPTIAINAKHQEHCTGTCPERIEHDDGWATFSKERTSNWGCEEFGCLAVETGCLFGSCQDVIRRELDVFSKLEEDKILTELCITLSHDTYCVTIDSTTPTINDYFEIQYKTVDVQTLPKMIGVTHHKLLRGQINELGSFGKFCGDIQVVGNQTYGQAAVKFDYICHAAQRKDVVIRKCLENNYQSCKLLTHDTDLILEESETSVEVINNKRITGQIALKVLLGDFNYKQYAANVEADIEANCVGCTNCIKGITCEIKVKTEIEASCKVEPPCPSYTNRIIIKPGRDTHTLLMKCDKKIMTGELAIKICNMQIQAHLSTIESNDQLELSTGDQSTYIHEEDLRCSTWICKVRDEGISFIFKPLTDWLGSFTKPILIAGCIIIVAIILIYILMPMCAKLRDLLKKNEYEYLQDTKVIVKPKATASSIGLRSKKINIQSSKAVD

SEQ ID NO: 96 - protein, 2275 aa, Umbre orthobunyavirus strain Marna
MLDQENEQALNRLAATVARANEPAEGKEAYNAILSRRHDYFGQVFCETIGIPYRNDVRLEDILHECDQTVDTLTNKIPNITPDNFEFRDNILTIIDYKVAVSDESADYTREKYENAVDAIKHLVDFPIRVCIVRIHPYTRQVTYSDDNFMRRFAHVVYPVDFTRYTQLTEELKEKFADSPEFMDMIAYGDVTFTANWCQNGCPELYEHPIFKEFLESMPLKYQKLFEKSLLSSCYTSERWDSNLKEVKAATKDEYEDFISRSAKQLYTTSPDYSEPSREEILKGWEEMTERVKEQREVSSNINDQKPSAHFIWAENNHELPTANSAKICAISKLLQSINIESSFAEDFKRLGKLFDFSEDIPGYERHCEQLKRQARSNPGQIKTKKLDPKKIGNALVLWEQQFLLSADEMGKENKLHLLKDFFGIGKHKQFARKGLDDTETDKPTILDFNDTEVKRSAELMMQKTKLYLSGKSSLNKEHPIASEYLNEIKKCNDETYNVLNAIFQTKYWQCITDISMLMKNMLSVSQYNRNNTFRIATCANNALYGLIFPSADIKTKDASIVYCIIAIHKDEKSLFNPGALHATFKVPGGFLSISKSMRLDKKRCHRIVTSPGIFLTIATMLKGDNPTISLNDVLNFSIFASLNITKSMLSLTEPSRYMIMNSLAVSSHVREYISEKFSPYTKTLFSVHMVEKIKAGCLNAFKQREKIKTRDIYLTDIDITQKGIQDNRDLCSIWFDGNVTLKEYLNQIYIVFYLNPKALHEKHHVMIDLLKTVIEIELDQRENVPQPWSDVPKKQTVKLPILVHSLAKNLLLDTSFAHFLRSRIESRNNFRRTFATISTFTSSKSCLKTGNFHEFKIKQCQRLKKVNASEAKKHRIANAMFVEEQDQHLEVEHANYELMRKAIPDYVDVLSTKVFDRLYELYKTGEIDDSPVIHQIFATMKSHTKFYFTYFNKGQKTAKDREIFVGEYEAKMCMYLVERIYKERSKVNPDEMISEPGDGKLRVLERKAEQEIRFMVEKMKAKNDEINKEIEDAKDNYVLNLGKIAALQAQKYKALKLEINADMSKWSAQDVFFKYFWSICLDPILYPEEKEHILYFFCNYMQKELVIPDEVICNILDQRKAYPNDIISQITNGLTTNHFNVKRNWLQGNFNYMSSYAHSTAMSVFKDVIKRAADLLEAEVLIHSMVHSDDNQTSVTLVDNRICPKQFTAFVINTFEKICLTFGCQANMKKTYITNHIKEFVSLFNLYGEPFSIYGRFTLTSVGDCAYIGPYEDLASRISATQTGIKHGCPASQAWLSIAIAQWMTYLTYNMLPGQQNDPQPILEIDRKQLPLELGGYISCPLSLIALAGLESGNIDFLIKLVNKYIDPRLQREPIQDQCTDIKNWDISKLSKVEIFKLKVLRYLVLDAEMDNTDIMGETSEMRGRSLLTPRKFTTAGSLRKLVSFEDFQAVQDSEQGVDSIVEYMLQNPALLVTKGETKDDYMNTVLYRYNSKKFKESLSIQNPTQLFLEQILFSHKPIVDYTGIAEKFSNLNDGTMLEDNPTIKGRMTFTDAFAMIKKDLSTLRITNEDLEIVLKFIILNDPLTVTAANAHILHVIGHSQPRLGSTACVMPEFRNLRMIKHSPALVLKCYSKNTLLLPGVQERDMERDLNHLKTFIETTRLEHKMQDRIKKNEDLKKSKDIYFEIKEVTRFYQTCYEYVKSTDYKVKVFILPAKCMTQTDFCAVLQGSLLEDKKWKLIQHLRPVTAGGHKGEVQPVVSMDFKLAREAVNLLCFFTDSFIDSRYRRDFLLKACVEMAYKDRPMVTLIEEIKKSKNRTSFLPFLYRIGELTQEDLDAYDAQKAGGRVTWNHWQSTRSLNMGKIDFQIDTHKTHLHIIGEDQQLVIAELKIPKLTANAITQAGYRLLNEKHGFRFETMNEVLVQPRKYYITYQMKSKKQYVYKIFDTATLLYERRNIKQYTGREANPIVAVCEVVPMEEEETPALSLSDIEMYNADNESVSILKTSFNESAKMRRANLSKMQYFETIGGSMLKIRFINVNALMKDTTLMSLNYDNLVNVDLARFSKLLDCDGDTESVEDGILCFSDDPMEQTTTEEIDAIPLFKVSYKISAPARLTYKNAIRELLRREITRFMDAFTFVGPSFDSPENMGFICNICCIIQLLHTNEWSIIMLNCIHICMIYLEKDIRFHKFLLNRIFFEGLNPASGKLDYKKIKEFVISLKDREMAPWNEIFSKFKQKCVTLLDKEITRIEQNTNFENILALDENTDDQSEFLLFE

SEQ ID NO: 97 - protein, 10 aa, artificial sequence
  synthetic peptide
GGWSHPQFEK